European Patent Application EP 4 316 487 A1, published February 7, 2024. Title: COMPOSITION FOR PREVENTING OR TREATING NEURODEGENERATIVE DISEASE COMPRISING COMPOUNDS THAT INDUCES THE EXPRESSION OF ANTI-AGING GENE KLOTHO. Applicant: Klotho Sciences. The sequence listing filed with the application follows.

SEQUENCE LISTING (4 sequences)

SEQ ID NO: 1 - DNA, 24 bp, Artificial Sequence
  KL-F
gatagagaaaaatggcttccctcc

SEQ ID NO: 2 - DNA, 24 bp, Artificial Sequence
  KL-R
ggtcggtaaactgagacagagtgg

SEQ ID NO: 3 - DNA, 24 bp, Artificial Sequence
  GAPDH-F
tgacaactttggtatcgtggaagg

SEQ ID NO: 4 - DNA, 22 bp, Artificial Sequence
  GAPDH-R
agggatgatgttctggagagcc